European Patent Application EP 4 190 818 A1, published June 7, 2023. Title: ANTI- HER2 ANTIBODY AND USE THEREOF. Applicant: Bio-Thera Solutions, Ltd. Application PCT/CN2021/108724. The sequence listing filed with the application follows.

SEQUENCE LISTING (13 sequences)

SEQ ID NO: 1 - protein, 8 aa, Artificial Sequence
GFTFTDYT

SEQ ID NO: 2 - protein, 15 aa, Artificial Sequence
VNPNSGGSIYNQRFK

SEQ ID NO: 3 - protein, 9 aa, Artificial Sequence
LGPSFYFDY

SEQ ID NO: 4 - protein, 11 aa, Artificial Sequence
KASQDVSIGVA

SEQ ID NO: 5 - protein, 7 aa, Artificial Sequence
ASYRYTG

SEQ ID NO: 6 - protein, 10 aa, Artificial Sequence
QQYYIYPYTF

SEQ ID NO: 7 - protein, 119 aa, Artificial Sequence [sequence omitted]

SEQ ID NO: 8 - protein, 108 aa, Artificial Sequence
DIQMTQSPSSLSASVGDRVTITCKASQDVSIGVAWYQQKPGKAPKLLIYSASYRYTGVPSRFSGSGSGTDFTLTISSLQPEDFATYYCQQYYIYPYTFGQGTKVEIKR

SEQ ID NO: 9 - protein, 449 aa, Artificial Sequence
EVQLVESGGGLVQPGGSLRLSCAASGFTFTDYTMDWVRQAPGKGLEWVADVNPNSGGSIYNQRFKGRFTLSVDRSKNTLYLQMNSLRAEDTAVYYCARNLGPSFYFDYWGQGTLVTVSSASTKGPSVFPLAPSSKSTSGGTAALGCLVKDYFPEPVTVSWNSGALTSGVHTFPAVLQSSGLYSLSSVVTVPSSSLGTQTYICNVNHKPSNTKVDKKVEPKSCDKTHTCPPCPAPELLGGPSVFLFPPKPKDTLMISRTPEVTCVVVDVSHEDPEVKFNWYVDGVEVHNAKTKPREEQYNSTYRVVSVLTVLHQDWLNGKEYKCKVSNKALPAPIEKTISKAKGQPREPQVYTLPPSREEMTKNQVSLTCLVKGFYPSDIAVEWESNGQPENNYKTTPPVLDSDGSFFLYSKLTVDKSRWQQGNVFSCSVMHEALHNHYTQKSLSLSPGK

SEQ ID NO: 10 - protein, 214 aa, Artificial Sequence
DIQMTQSPSSLSASVGDRVTITCKASQDVSIGVAWYQQKPGKAPKLLIYSASYRYTGVPSRFSGSGSGTDFTLTISSLQPEDFATYYCQQYYIYPYTFGQGTKVEIKRTVAAPSVFIFPPSDEQLKSGTASVVCLLNNFYPREAKVQWKVDNALQSGNSQESVTEQDSKDSTYSLSSTLTLSKADYEKHKVYACEVTHQGLSSPVTKSFNRGEC

SEQ ID NO: 11 - protein, 636 aa, Artificial Sequence
TQVCTGTDMKLRLPASPETHLDMLRHLYQGCQVVQGNLELTYLPTNASLSFLQDIQEVQGYVLIAHNQVRQVPLQRLRIVRGTQLFEDNYALAVLDNGDPLNNTTPVTGASPGGLRELQLRSLTEILKGGVLIQRNPQLCYQDTILWKDIFHKNNQLALTLIDTNRSRACHPCSPMCKGSRCWGESSEDCQSLTRTVCAGGCARCKGPLPTDCCHEQCAAGCTGPKHSDCLACLHFNHSGICELHCPALVTYNTDTFESMPNPEGRYTFGASCVTACPYNYLSTDVGSCTLVCPLHNQEVTAEDGTQRCEKCSKPCARVCYGLGMEHLREVRAVTSANIQEFAGCKKIFGSLAFLPESFDGDPASNTAPLQPEQLQVFETLEEITGYLYISAWPDSLPDLSVFQNLQVIRGRILHNGAYSLTLQGLGISWLGLRSLRELGSGLALIHHNTHLCFVHTVPWDQLFRNPHQALLHTANRPEDECVGEGLACHQLCARGHCWGPGPTQCVNCSQFLRGQECVEECRVLQGLPREYVNARHCLPCHPECQPQNGSVTCFGPEADQCVACAHYKDPPFCVARCPSGVKPDLSYMPIWKFPDEEGACQPCPINCTHSCVDLDDKGCPAEQRASPLTHHHHHH

SEQ ID NO: 12 - DNA, 642 bp, Artificial Sequence
gatatccagatgacccagagcccttcctccctgagcgctagcgtgggcgaccgggtgaccatcacctgcaaggctagccaggacgtgtccatcggcgtggcctggtaccagcagaagcccggcaaggcccccaagctgctgatctactccgcttcctatcggtataccggcgtgccttccaggttctccggcagcggctccggcaccgacttcaccctgaccatctcctccctgcagcctgaggacttcgccacctactactgtcagcagtactacatctacccttacaccttcggccagggcaccaaggtggagatcaaacgtacggtggctgcaccatctgtcttcatcttcccgccatctgatgagcagttgaaatctggaactgcctctgttgtgtgcctgctgaataacttctatcccagagaggccaaagtacagtggaaggtggataacgccctccaatcgggtaactcccaggagagtgtcacagagcaggacagcaaggacagcacctacagcctcagcagcaccctgacgctgagcaaagcagactacgagaaacacaaagtctacgcctgcgaagtcacccatcagggcctgagctcgcccgtcacaaagagcttcaacaggggagagtgt

SEQ ID NO: 13 - DNA, 1347 bp, Artificial Sequence
gaggtgcagctggtggagtccggcggcggactggtgcagccaggaggaagcctgaggctgtcctgcgccgctagcggcttcaccttcaccgattacaccatggactgggtgaggcaggcccctggcaagggcctggagtgggtggctgacgtgaatcccaatagcggcggctccatctacaatcagaggttcaagggcaggtttaccctgtccgtggataggagcaagaataccctgtacctgcagatgaactccctgagggccgaggacaccgccgtgtattattgtgctcggaatctgggccctagcttttatttcgattattggggccagggtaccctggtcaccgtgtctagtgctagtactaaggggccttcagtgtttccactggcaccctcatccaaatccaccagcggcggaacagcagccctgggttgtctggtgaaggactacttcccagaacccgtcaccgtgtcatggaactccggcgcactgacatctggagtccacacttttcctgccgtgctgcagagctctgggctgtactccctgagttcagtggtcactgtcccatccagctctctgggtacacagacttatatctgcaacgtgaatcacaagccaagtaataccaaagtcgacaagaaagtggagcccaagtcatgtgataaaacccatacatgccccccttgtcctgcaccagaactgctgggaggtccaagcgtgttcctgtttccacccaagcctaaagacacactgatgattagtaggactcccgaggtcacctgcgtggtcgtggacgtgtcccacgaggatcctgaagtcaagtttaactggtacgtggatggcgtcgaagtgcataatgctaagaccaaaccaagagaggaacagtacaactccacttatcgcgtcgtgagcgtcctgaccgtgctgcatcaggattggctgaacggcaaggagtataagtgcaaagtgagcaataaggctctgcccgcacctatcgagaaaaccatttctaaggcaaaaggacagcctcgagaaccacaggtgtacacactgcctccaagccgtgaggaaatgaccaagaaccaggtctctctgacatgtctggtgaaaggcttctatccttcagacattgctgtggagtgggaatccaatggacagccagagaacaattacaagaccacaccccctgtgctggacagcgatggctctttctttctgtattctaagctgaccgtggataaaagtcggtggcagcagggaaatgtcttttcttgtagtgtgatgcacgaagcactgcacaaccactacacccagaaatcactgtcactgtctccagggaag